European Patent Specification EP 3 773 910 B1, published July 24, 2024. Title: Novel Anti-Prostate-Specific Membrane Antigen (PSMA) Antibody Drug Conjugates. Applicant: Ambrx, Inc. The sequence listing filed with the application follows.

SEQUENCE LISTING (17 sequences)

SEQ ID NO: 1 - protein, 115 aa, Artificial Sequence
  Humanized Heavy Chain Variable Region
QVQLVQSGAEVKKPGASVKVSCKASGYTFTEYTIHWVRQAPGQRLEWMGNINPNNGGTTYNQKFEDRVTITRDTSASTAYMELSSLRSEDTAVYYCAAGWNFDYWGQGTTLTVSS

SEQ ID NO: 2 - protein, 110 aa, Artificial Sequence
  Humanized Light Chain Variable Region
DIQLTQSPSFLSASVGDRVTITCKASQDVGTAVDWYQQKPGKAPKLLIYWASTRHTGVPSRFSGSGSGTEFTLTISSLQPEDFATYYCQQYNSYPLTFGGGTKVEIKRTV

SEQ ID NO: 3 - protein, 110 aa, Artificial Sequence
  Humanized Light Chain Variable Region
DIQLTQSPSFLSASVGDRVTITCKASQDVGTAVDWYQQKPGKAPKLLIYWASTRHTGVPDRFSGSGSGTEFTLTISSLQPEDFATYYCQQYNSYPLTFGGGTKVEIKRTV

SEQ ID NO: 4 - protein, 110 aa, Artificial Sequence
  Humanized Light Chain Variable Region
DIQLTQSPSFLSASVGDRVTITCKASQDVGTAVDWYQQKPGKAPKLLIYWASTRHTGVPSRFSGSGSGTEFTLTISSLQSEDFATYYCQQYNSYPLTFGGGTKVEIKRTV

SEQ ID NO: 5 - protein, 110 aa, Artificial Sequence
  Humanized Light Chain Variable Region
DIQLTQSPSFLSASVGDRVTITCKASQDVGTAVDWYQQKPGKAPKLLIYWASTRHTGVPSRFSGSGSGTEFTLTISNLQPEDFATYYCQQYNSYPLTFGGGTKVEIKRTV

SEQ ID NO: 6 - protein, 115 aa, Artificial Sequence
  Chimeric Heavy Chain Variable Region
EVQLQQSGPELVKPGTSVRISCKTSGYTFTEYTIHWVKQSHGKSLEWIGNINPNNGGTTYNQKFEDKATLTVDKSSSTAYMELRSLTSEDSAVYYCAAGWNFDYWGQGTTLTVSS

SEQ ID NO: 7 - protein, 110 aa, Artificial Sequence
  Chimeric Light Chain Variable Region
DIVMTQSHKFMSTSVGDRVSIICKASQDVGTAVDWYQQKPGQSPKLLIYWASTRHTGVPDRFTGSGSGTDFTLTITNVQSEDLADYFCQQYNSYPLTFGAGTKVEIKRTV

SEQ ID NO: 8 - protein, 444 aa, Artificial Sequence
  Humanized Anti-PSMA Variant - Heavy Chain
QVQLVQSGAEVKKPGASVKVSCKASGYTFTEYTIHWVRQAPGQRLEWMGNINPNNGGTTYNQKFEDRVTITRDTSASTAYMELSSLRSEDTAVYYCAAGWNFDYWGQGTTLTVSSASTKGPSVFPLAPSSKSTSGGTAALGCLVKDYFPEPVTVSWNSGALTSGVHTFPAVLQSSGLYSLSSVVTVPSSSLGTQTYICNVNHKPSNTKVDKKVEPKSCDKTHTCPPCPAPELLGGPSVFLFPPKPKDTLMISRTPEVTCVVVDVSHEDPEVKFNWYVDGVEVHNAKTKPREEQYNSTYRVVSVLTVLHQDWLNGKEYKCKVSNKALPAPIEKTISKAKGQPREPQVYTLPPSRDELTKNQVSLTCLVKGFYPSDIAVEWESNGQPENNYKTTPPVLDSDGSFFLYSKLTVDKSRWQQGNVFSCSVMHEALHNHYTQKSLSLSPG

SEQ ID NO: 9 - protein, 214 aa, Artificial Sequence
  Humanized Anti-PSMA Variant - Light Chain
DIQLTQSPSFLSASVGDRVTITCKASQDVGTAVDWYQQKPGKAPKLLIYWASTRHTGVPSRFSGSGSGTEFTLTISSLQPEDFATYYCQQYNSYPLTFGGGTKVEIKRTVAAPSVFIFPPSDEQLKSGTASVVCLLNNFYPREAKVQWKVDNALQSGNSQESVTEQDSKDSTYSLSSTLTLSKADYEKHKVYACEVTHQGLSSPVTKSFNRGEC

SEQ ID NO: 10 - protein, 444 aa, Artificial Sequence; identical to SEQ ID NO: 8
  Humanized Anti-PSMA Variant - Heavy Chain

SEQ ID NO: 11 - protein, 214 aa, Artificial Sequence
  Humanized Anti-PSMA Variant - Light Chain
DIQLTQSPSFLSASVGDRVTITCKASQDVGTAVDWYQQKPGKAPKLLIYWASTRHTGVPSRFSGSGSGTEFTLTISSLQSEDFATYYCQQYNSYPLTFGGGTKVEIKRTVAAPSVFIFPPSDEQLKSGTASVVCLLNNFYPREAKVQWKVDNALQSGNSQESVTEQDSKDSTYSLSSTLTLSKADYEKHKVYACEVTHQGLSSPVTKSFNRGEC

SEQ ID NO: 12 - protein, 444 aa, Artificial Sequence; identical to SEQ ID NO: 8
  Humanized Anti-PSMA Variant - Heavy Chain

SEQ ID NO: 13 - protein, 214 aa, Artificial Sequence
  Humanized Anti-PSMA Variant - Light Chain
DIQLTQSPSFLSASVGDRVTITCKASQDVGTAVDWYQQKPGKAPKLLIYWASTRHTGVPDRFSGSGSGTEFTLTISSLQPEDFATYYCQQYNSYPLTFGGGTKVEIKRTVAAPSVFIFPPSDEQLKSGTASVVCLLNNFYPREAKVQWKVDNALQSGNSQESVTEQDSKDSTYSLSSTLTLSKADYEKHKVYACEVTHQGLSSPVTKSFNRGEC

SEQ ID NO: 14 - protein, 444 aa, Artificial Sequence; identical to SEQ ID NO: 8
  Humanized Anti-PSMA Variant - Heavy Chain

SEQ ID NO: 15 - protein, 214 aa, Artificial Sequence
  Humanized Anti-PSMA Variant - Light Chain
DIQLTQSPSFLSASVGDRVTITCKASQDVGTAVDWYQQKPGKAPKLLIYWASTRHTGVPSRFSGSGSGTEFTLTISNLQPEDFATYYCQQYNSYPLTFGGGTKVEIKRTVAAPSVFIFPPSDEQLKSGTASVVCLLNNFYPREAKVQWKVDNALQSGNSQESVTEQDSKDSTYSLSSTLTLSKADYEKHKVYACEVTHQGLSSPVTKSFNRGEC

SEQ ID NO: 16 - protein, 444 aa, Artificial Sequence
  Chimeric Anti-PSMA Antibody Variant - Heavy Chain
EVQLQQSGPELVKPGTSVRISCKTSGYTFTEYTIHWVKQSHGKSLEWIGNINPNNGGTTYNQKFEDKATLTVDKSSSTAYMELRSLTSEDSAVYYCAAGWNFDYWGQGTTLTVSSASTKGPSVFPLAPSSKSTSGGTAALGCLVKDYFPEPVTVSWNSGALTSGVHTFPAVLQSSGLYSLSSVVTVPSSSLGTQTYICNVNHKPSNTKVDKKVEPKSCDKTHTCPPCPAPELLGGPSVFLFPPKPKDTLMISRTPEVTCVVVDVSHEDPEVKFNWYVDGVEVHNAKTKPREEQYNSTYRVVSVLTVLHQDWLNGKEYKCKVSNKALPAPIEKTISKAKGQPREPQVYTLPPSRDELTKNQVSLTCLVKGFYPSDIAVEWESNGQPENNYKTTPPVLDSDGSFFLYSKLTVDKSRWQQGNVFSCSVMHEALHNHYTQKSLSLSPG

SEQ ID NO: 17 - protein, 190 aa, Artificial Sequence
  Chimeric Anti-PSMA Antibody Variant - Light Chain
DIVMTQSHKFMSTSVGDRVSIICKASQDVGTAVDWYQQKPGQSPKLLIYWASTRHTGVPDRFTGSGSGTDFTLTITNVQSEDLADYFCQQYNSYPLTFGAGTKVEIKRTVAAPSVFIFPPSDEQLKSGTASVVCLLNNFYPREAKVQWKVDNALQSGNSQESVTEQDSKDSTYSLSSTLTLSKADYEKHK